European Patent Application EP 4 310 095 A1, published January 24, 2024. Title: Follicular helper T cells (Tfh) specific for SARS-CoV-2 virus. Applicant: Osaka University KOTAI Biotechnologies, Inc. The sequence listing filed with the application follows.

SEQUENCE LISTING (56 sequences)

SEQ ID NO: 1 - protein, 19 aa, artificial sequence
  amino acid sequence of S864 - S882 of SARS-CoV-2
LLTDEMIAQYTSALLAGTI

SEQ ID NO: 2 - protein, 13 aa, artificial sequence
  amino acid sequence of CDR3 alpha of clone 1 and 2
CVVNRGSSYKLIF

SEQ ID NO: 3 - protein, 11 aa, artificial sequence
  amino acid sequence of CDR3 beta of clone 1
CASSQTYEQYF

SEQ ID NO: 4 - protein, 10 aa, artificial sequence
  amino acid sequence of CDR3 beta of clone 2
CASSPTYEQY

SEQ ID NO: 5 - protein, 9 aa, artificial sequence
  amino acid sequence of epitope of SARS-CoV-2 for focillar helper T cell
  misc_feature (1)..(9): Xaa can be any naturally occurring amino acid
XXXXXXXXX

SEQ ID NO: 6 - protein, 9 aa, artificial sequence
  amino acid sequence of epitope of SARS-CoV-2 for focillar helper T cell
  misc_feature (1)..(1): Xaa can be any naturally occurring amino acid
XAQYTSALL

SEQ ID NO: 7 - protein, 9 aa, artificial sequence
  amino acid sequence of epitope of SARS-CoV-2 for focillar helper T cell
  misc_feature (2)..(2): Xaa can be any naturally occurring amino acid
IXQYTSALL

SEQ ID NO: 8 - protein, 10 aa, artificial sequence
  amino acid sequence of epitope of SARS-CoV-2 for focillar helper T cell
  misc_feature (4)..(4): Xaa can be any naturally occurring amino acid
IAQXYTSALL

SEQ ID NO: 9 - protein, 9 aa, artificial sequence
  amino acid sequence of epitope of SARS-CoV-2 for focillar helper T cell
  misc_feature (6)..(6): Xaa can be any naturally occurring amino acid
IAQYTXALL

SEQ ID NO: 10 - protein, 9 aa, artificial sequence
  amino acid sequence of epitope of SARS-CoV-2 for focillar helper T cell
  misc_feature (7)..(7): Xaa can be any naturally occurring amino acid
IAQYTSXLL

SEQ ID NO: 11 - protein, 9 aa, artificial sequence
  amino acid sequence of epitope of SARS-CoV-2 for focillar helper T cell
  misc_feature (8)..(8): Xaa can be any naturally occurring amino acid
IAQYTSAXL

SEQ ID NO: 12 - protein, 9 aa, artificial sequence
  amino acid sequence of epitope of SARS-CoV-2 for focillar helper T cell
  misc_feature (9)..(9): Xaa can be any naturally occurring amino acid
IAQYTSALX

SEQ ID NO: 13 - protein, 9 aa, artificial sequence
  amino acid sequence of epitope of SARS-CoV-2 for focillar helper T cell
IAQYTSALL

SEQ ID NO: 14 - protein, 14 aa, artificial sequence
  amino acid sequence of CDR3 alpha of clone 1-1
CVVSRTGGGNKLTF

SEQ ID NO: 15 - protein, 15 aa, artificial sequence
  amino acid sequence of CDR3 beta of clone 1-1
CASSQAGGSTDTQYF

SEQ ID NO: 16 - protein, 12 aa, artificial sequence
  amino acid sequence of CDR3 alpha of clone 1-2
CAALNAGNMLTF

SEQ ID NO: 17 - protein, 14 aa, artificial sequence
  amino acid sequence of CDR3 alpha of clone 2
CVVNKGSSASKIIF

SEQ ID NO: 18 - protein, 14 aa, artificial sequence
  amino acid sequence of CDR3 beta of clone 2
CASSEGASNQPQHF

SEQ ID NO: 19 - protein, 14 aa, artificial sequence
  amino acid sequence of CDR3 alpha of clone 3-1
CAMTYSGGYQKVTF

SEQ ID NO: 20 - protein, 13 aa, artificial sequence
  amino acid sequence of CDR3 brta of clone 3-1
CSARAGVQETQYF

SEQ ID NO: 21 - protein, 14 aa, artificial sequence
  amino acid sequence of CDR3 alpha of clone 3-2
CAMTPSGGYQKVTF

SEQ ID NO: 22 - protein, 14 aa, artificial sequence
  amino acid sequence of CDR3 alpha of clone 4
CAVSDQGRDDKIIF

SEQ ID NO: 23 - protein, 13 aa, artificial sequence
  amino acid sequence of CDR3 beta of clone 4
CSARDWREETQYF

SEQ ID NO: 24 - protein, 11 aa, artificial sequence
  amino acid sequence of CDR3 beta of clone 5-2
CASSPTYEQYF

SEQ ID NO: 25 - protein, 14 aa, artificial sequence
  amino acid sequence of CDR3 alpha of clone 6
CAENSGGSNYKLTF

SEQ ID NO: 26 - protein, 14 aa, artificial sequence
  amino acid sequence of CDR3 beta of clone 6
CSAKTSGRGETQYF

SEQ ID NO: 27 - protein, 16 aa, artificial sequence
  amino acid sequence of CDR3 alpha of clone 7-1
CAATLYSGAGSYQLTF

SEQ ID NO: 28 - protein, 12 aa, artificial sequence
  amino acid sequence of CDR3 beta of clone 7-1
CASSSREDTQYF

SEQ ID NO: 29 - protein, 16 aa, artificial sequence
  amino acid sequence of CDR3 alpha of clone 7-2
CAATSYSGAGSYQLTF

SEQ ID NO: 30 - protein, 17 aa, artificial sequence
  amino acid sequence of CDR3 alpha of clone 8
CAASPPSYGGSQGNLIF

SEQ ID NO: 31 - protein, 13 aa, artificial sequence
  amino acid sequence of CDR3 beta of clone 8
CSVYRGLDEKLFF

SEQ ID NO: 32 - protein, 14 aa, artificial sequence
  amino acid sequence of CDR3 alpha of clone 9
CALSGGNRDDKIIF

SEQ ID NO: 33 - protein, 13 aa, artificial sequence
  amino acid sequence of CDR3 beta of clone 9
CSARDWRGETQYF

SEQ ID NO: 34 - protein, 9 aa, artificial sequence
  amino acid sequence of CDR3 alpha of clone 10-1
CAAQYALNF

SEQ ID NO: 35 - protein, 15 aa, artificial sequence
  amino acid sequence of CDR3 beta of clone 10-2
CASSHGTGGRYEQYF

SEQ ID NO: 36 - protein, 9 aa, artificial sequence
  amino acid sequence of CDR3 alpha of clone 10-2
CAAGYALNF

SEQ ID NO: 37 - protein, 15 aa, artificial sequence
  amino acid sequence of CDR3 beta of clone 10-2
CASSLGTSGRYEQYF

SEQ ID NO: 38 - protein, 7 aa, artificial sequence
  amino acid sequence of epitope of SARS-CoV-2 for focillar helper T cell
LLQYGSF

SEQ ID NO: 39 - protein, 15 aa, artificial sequence
  amino acid sequence of epitope of SARS-CoV-2 for focillar helper T cell
WNRKRISNCVADYSV

SEQ ID NO: 40 - protein, 11 aa, artificial sequence
  amino acid sequence of epitope of SARS-CoV-2 for focillar helper T cell
FIKQYGDCLGD

SEQ ID NO: 41 - protein, 11 aa, artificial sequence
  amino acid sequence of epitope of SARS-CoV-2 for focillar helper T cell
MIAQYTSALLA

SEQ ID NO: 42 - protein, 11 aa, artificial sequence
  amino acid sequence of epitope of SARS-CoV-2 for focillar helper T cell
KKFLPFQQFGR

SEQ ID NO: 43 - protein, 11 aa, artificial sequence
  amino acid sequence of epitope of SARS-CoV-2 for focillar helper T cell
QALNTLVKQLS

SEQ ID NO: 44 - protein, 15 aa, artificial sequence
  amino acid sequence of a part of SARS-CoV-2 protein
LPPLLTDEMIAQYTS

SEQ ID NO: 45 - protein, 15 aa, artificial sequence
  amino acid sequence of a part of SARS-CoV-2 protein
PPLLTDEMIAQYTSA

SEQ ID NO: 46 - protein, 15 aa, artificial sequence
  amino acid sequence of a part of SARS-CoV-2 protein
PLLTDEMIAQYTSAL

SEQ ID NO: 47 - protein, 15 aa, artificial sequence
  amino acid sequence of a part of SARS-CoV-2 protein
LLTDEMIAQYTSALL

SEQ ID NO: 48 - protein, 15 aa, artificial sequence
  amino acid sequence of a part of SARS-CoV-2 protein
LTDEMIAQYTSALLA

SEQ ID NO: 49 - protein, 15 aa, artificial sequence
  amino acid sequence of a part of SARS-CoV-2 protein
TDEMIAQYTSALLAG

SEQ ID NO: 50 - protein, 15 aa, artificial sequence
  amino acid sequence of a part of SARS-CoV-2 protein
DEMIAQYTSALLAGT

SEQ ID NO: 51 - protein, 15 aa, artificial sequence
  amino acid sequence of a part of SARS-CoV-2 protein
EMIAQYTSALLAGTI

SEQ ID NO: 52 - protein, 15 aa, artificial sequence
  amino acid sequence of a part of SARS-CoV-2 protein
MIAQYTSALLAGTIT

SEQ ID NO: 53 - protein, 15 aa, artificial sequence
  amino acid sequence of a part of SARS-CoV-2 protein
IAQYTSALLAGTITS

SEQ ID NO: 54 - protein, 15 aa, artificial sequence
  amino acid sequence of a part of SARS-CoV-2 protein
AQYTSALLAGTITSG

SEQ ID NO: 55 - protein, 15 aa, artificial sequence
  amino acid sequence of a part of SARS-CoV-2 protein
QYTSALLAGTITSGW

SEQ ID NO: 56 - protein, 15 aa, artificial sequence
  amino acid sequence of a part of SARS-CoV-2 protein
YTSALLAGTITSGWT